European Patent Application EP 4 242 301 A1, published September 13, 2023. Title: COMPOUND ENZYME AND APPLICATION THEREOF IN PREPARATION OF L-ERGOTHI ONEINE. Applicant: Shenzhen Readline Biotechnology Co., Ltd. The sequence listing filed with the application follows.

SEQUENCE LISTING (16 sequences)

SEQ ID NO: 1 - protein, 321 aa, Mycobacterium smegmatis
MTLSLANYLAADSAAEALRRDVRAGLTAAPKSLPPKWFYDAVGSDLFDQITRLPEYYPTRTEAQILRTRSAEIIAAAGADTLVELGSGTSEKTRMLLDAMRDAELLRRFIPFDVDAGVLRSAGAAIGAEYPGIEIDAVCGDFEEHLGKIPHVGRRLVVFLGSTIGNLTPAPRAEFLSTLADTLQPGDSLLLGTDLVKDTGRLVRAYDDAAGVTAAFNRNVLAVVNRELSADFDLDAFEHVAKWNSDEERIEMWLRARTAQHVRVAALDLEVDFAAGEEMLTEVSCKFRPENVVAELAEAGLRQTHWWTDPAGDFGLSLAVR

SEQ ID NO: 2 - protein, 333 aa, Chlorobium limicola
MAYSKTNLSELPLADIDNHLTEIGFDTTISEIITGLTANAKYIQSKYFYDKRGSALFEKITSLSEYYPSRTEKAIISQLPPALIEDLADIDIIELGCGDHSKISLLIRRIPAESVPGLRYFPIDISQTALKQSIEDLRDLFPALKVKGILADYVHQMHLFPEERKRLFCFFGSTIGNLSREETLDFMQNMGTTMHPGDMLLVGMDRVKNIALLEKAYNDDQFITAMFNKNILRVINGLIKSDFNPDDFEHRAFYNADFNRIEMHLEATGNISVKSAFMPELIRIKKGETIHTENSHKFEKADILLMGQHAGLAIKNIYSDKNELFSLAHYEKK

SEQ ID NO: 3 - protein, 199 aa, Chloracidobacterium thermophilum
MLGMDADTASFWEEKYRADLTAWDRGGVSPALEHWLAEGALKPGRILIPGCGYGHEVLALARRGFEVWGLDIALTPVRRLQEKLAQAGLTAHVVEGDVRTWQPEQPFDAVYEQTCLCALSPEDWPRYEAQLCRWLRPGGRLFALWMQTDRPGGPPYHCGLEAMRVLFALERWRWVEPPQRTVPHPTGFFEYAAILERLV

SEQ ID NO: 4 - protein, 199 aa, Methylibium sp
MSGPDLNFWQQRFDAGQLPWDRGAPSPQLAAWLGDGSLKPGRIAVPGCGSGHEVVALARGGFSVTAIDYAPGAVRLTQGRLAAAGLAAEVVQADVLTWQPTAPLDAVYEQTCLCALHPDHWVAYFARLHAWLRPGGTLALLAMQALRESAGQGLIEGPPYHVDVNALRALLPGDRWDWPRPPYARVPHPSSTWQNWPSC

SEQ ID NO: 5 - protein, 457 aa, Chlorobium limicola
MQNKNFRAPQSEAIGILYKLIETGSKHKNMYDHTEITTDSLLALLGSEKVKIIDVRSADAYNGWRMRGEVRGGHIKGAKSLPAKWLTDPEWLNIVRFKQIRPEDAIVLYGYTPEECEQTATRFKENGYNNVSVFHRFHPDWTGNDAFPMDRLEQYNRLVPAEWVNGLISGEEIPEYDNDTFIVCHAHYRNRDAYLSGHIPGATDMDTLALESPETWNRRTPEELKKALEEHGITASTTVVLYGKFMHPDNADEFPGSAAGHIGAIRLAFIMMYAGVEDVRVLNGGYQSWTDAGFAISKDDVPKTTVPEFGAPIPSRPEFAVDIDEAKEMLQSEDSDLVCVRSYPEYIGEVSGYNYIKKKGRIPGAIFAECGSDAYHMENYRNHDHTTREYHEIEDIWAKSGIIPKKHLAFYCGTGWRGSEAWFNALLMGWPRVSVYDGGWFEWSNDPENPYETGVPK

SEQ ID NO: 6 - protein, 440 aa, Escherichia coli
MSGFSMKRVSQMTALAMALGLACASSWAAELAKPLTLDQLQQQNGKAIDTRPSAFYNGWPQTLNGPSGHEPAALNLSASWLDKMSTEQLNEWIKQHNLKADAPVALYGNDKDVDAVKTRLQKAGFTHISILSDALSEPSRLQKLPHFEQLVYPQWLHNLQQGKEVTAKPAGDWKVIEAAWGAPKFYLISHIPGADYIDTNEVESEPLWNKVSDEQLKAMLAKHGIRHDTTVILYGRDVYAAARVAQIMLYAGVKDVRLLDGGWQTWSDAGLPVERGTPPKVKAEPDFGVKIPAQPQLMLDMEQARGLLHRQDASLVSIRSWPEFIGTTSGYSYIKPKGEIAGARWGHAGSDSTHMEDFHNPDGTMRSADDITAMWKAWNIKPDQQVSFYCGTGWRASETFMYARAMGWNNVSVYDGGWYEWSSDPKNPVATGERGPDSSK

SEQ ID NO: 7 - DNA, 966 bp, Artificial Sequence
  MsHisMT
atgacgctctcactggccaactacctggcagccgactcggccgccgaagcactgcgccgtgacgtccgcgcgggcctcaccgcggcaccgaagagtctgccgcccaagtggttctacgacgccgtcggcagtgatctgttcgaccagatcacccggctccccgagtattaccccacccgcaccgaggcgcagatcctgcggacccggtcggcggagatcatcgcggccgcgggtgccgacaccctggtggaactgggcagtggtacgtcggagaaaacccgcatgctgctcgacgccatgcgcgacgccgagttgctgcgccgcttcatcccgttcgacgtcgacgcgggcgtgctgcgctcggccggggcggcaatcggcgcggagtaccccggtatcgagatcgacgcggtatgtggcgatttcgaggaacatctgggcaagatcccgcatgtcggacggcggctcgtggtgttcctggggtcgaccatcggcaacctgacacccgcgccccgcgcggagttcctcagtactctcgcggacacgctgcagccgggcgacagcctgctgctgggcaccgatctggtgaaggacaccggccggttggtgcgcgcgtacgacgacgcggccggcgtcaccgcggcgttcaaccgcaacgtgctggccgtggtgaaccgcgaactgtccgccgatttcgacctcgacgcgttcgagcatgtcgcgaagtggaactccgacgaggaacgcatcgagatgtggttgcgtgcccgcaccgcacagcatgtccgcgtcgcggcactggacctggaggtcgacttcgccgcgggtgaggagatgctcaccgaggtgtcctgcaagttccgtcccgagaacgtcgtcgccgagctggcggaagccggtctgcggcagacgcattggtggaccgatccggccggggatttcgggttgtcgctggcggtgcggtga

SEQ ID NO: 8 - DNA, 1002 bp, Artificial Sequence
  ClHisMT
atggcatactcgaagaccaatctttccgaactgccccttgcggacatagacaaccatttaactgagataggcttcgacactactatttcagagattattactgggttgactgctaatgcgaagtatattcagtccaagtacttttatgataaacggggttctgctttatttgagaaaattacttcattatcagagtactacccgagtagaacagagaaggctataatttcacaattaccgccagccttaatagaagatctggctgacatcgacattatcgagttgggctgcggagatcacagcaagatctcactgcttatacgccggatacccgccgaatctgtgcctggtttgcgctatttcccaattgatatctctcaaacggctttaaaacaatcaatcgaggacttgagagacttatttccagccctgaaggttaaaggcatccttgcagattatgttcaccagatgcacctgttcccagaggaacgtaaacgcttgttttgtttctttggttctacgataggcaatctgtcacgtgaagagacactggattttatgcagaacatgggcacaactatgcacccaggcgatatgttactggtcggtatggatcgtgtaaagaatatcgcattactggagaaggcatataatgacgatcaattcataacggcaatgtttaacaaaaatatattgcgcgttataaacggattaataaaatctgacttcaatcctgacgatttcgagcaccgtgctttttataatgcggactttaacagaatcgaaatgcaccttgaagctaccggtaatatctcggtgaagagcgcattcatgccagaactgatacggattaaaaaaggagaaactatccacacagagaacagtcacaaatttgagaaagctgatatattgttaatgggacagcatgcagggttagcgatcaagaacatctattccgacaagaacgaactttttagcctggcccattatgagaagaagtga

SEQ ID NO: 9 - DNA, 600 bp, Artificial Sequence
  CtHaMT
atgctgggcatggacgctgatactgcgagcttctgggaagagaaatatcgcgccgacttaaccgcatgggatcggggcggtgtatctcccgctctggaacattggttggccgagggtgcgttgaaacccggtcgcattttgataccgggctgcgggtatggccacgaagtcttagctttagctcggcgcggatttgaggtttgggggcttgacatagcactgacacccgttcgtcggcttcaagaaaagttggcacaggctggtcttacggcacacgtagtcgagggcgacgtgcgtacttggcaacccgaacaaccgttcgatgcagtatatgaacaaacatgcttatgcgcccttagccccgaagattggccacggtacgaagcccaattgtgccgttggcttagacctggcggcagattattcgcactttggatgcagacagaccggccaggcggaccgccataccattgtgggttggaagcaatgcgtgttttatttgcgcttgaaagatggcgttgggtcgaaccgccccagagaacagtgccacaccctacaggtttcttcgagtatgccgcgatccttgaacggttggtctga

SEQ ID NO: 10 - DNA, 612 bp, Artificial Sequence
  MspHaMT
atgagtggacccgacttaaatttctggcagcaacgttttgacaccggccaacttccgtgggaccgtggcgcaccttcgccacaactggcggcttggttgggtgatgggtcattagcgccaggtcgcattgccgtaccggggtgcggttcaggacatgaagttgttgcgttagcccgcggtgggttctcagtaacagccattgattacgcccccggagcagtgcgcttaacccaaggccgcttggctgcggcggggttagcggcggaagtcgtgcaggctgacgtacttacgtggcagccaacggctccgcttgacgctgtgtacgagcaaacttgtctgtgtgcattgcatcccgaccattgggtggcatacgcagctagattacacgcttggcttagaccaggaggtactttggcattgttggcaatgcaggcactgcgtgagggcgctggacagggcttgatagaagggcctccttaccatgttgacgttaacgctcttcgcgcgctgctgccgggggaccgttgggactggccacgtccaccgtatgcgcgcgttcctcacccctcttctacatgggccgagttggcaatagtcctgactcggcgttga

SEQ ID NO: 11 - DNA, 1374 bp, Artificial Sequence
  ClHerS
atgcagaataagaattttcgtgcaccccagtcagaggccataggcatcttgtataaacttattgaaactggatcgaagcacaaaaacatgtacgaccacacagagatcacaacagacagtctgttggcacttttgggttcggaaaaggtgaagataattgacgttcgctcggctgacgcgtataacggttggcggatgcgtggtgaagtacgtggaggccacatcaaaggtgcaaagtcgttgccagcgaagtggctgacagatccggaatggcttaacattgttcgtttcaaacagatacgtcccgaggacgccatcgtcctttatggttatacgcccgaggagtgcgaacaaactgccactagattcaaagagaatggttataataatgtgagcgtatttcacagattccacccggactggactgggaacgatgctttcccaatggatagactggagcaatataatagacttgtacccgccgaatgggttaacggtttgataagcggggaagagatcccagagtacgacaatgacaccttcatcgtgtgtcatgcacattatcggaacagagatgcgtatcttagcggccacattccgggtgctactgacatggatactttggcgttagaatcgccagagacctggaatcgtcggactccagaagaattaaagaaagctttagaagagcatgggataacggcttcgacgactgtcgttctttatgggaaatttatgcatcccgataacgcagatgaatttcctggatccgcagctggccatatcggggcgattcgcttggctttcattatgatgtacgcgggggttgaggacgttcgggtcctgaatggcgggtatcaatcatggaccgatgcgggatttgctatttccaaagatgacgtgccaaagacgactgtcccagagttcggcgcacccattccttcccgtccggaattcgctgtagatatcgacgaagccaaggaaatgcttcaatcagaggattcagatctggtgtgcgtgcgctcgtacccggagtatatcggcgaggtcagcggctataattacataaaaaaaaagggcagaatcccgggggctatatttgctgagtgcgggtcggatgcctatcacatggaaaactatagaaatcatgaccacaccacgcgcgaatatcatgaaatagaagatatatgggcaaaaagcgggatcatcccgaagaaacacttggctttttattgcggtactggatggcgtggttctgaggcttggttcaacgcgttgctgatgggttggccgcgcgtttccgtttatgacggcggttggtttgagtggagcaacgaccccgaaaacccatacgagacgggagttccgaagtga

SEQ ID NO: 12 - DNA, 1323 bp, Artificial Sequence
  EcHerS
atgtcgggattttcgatgaaacgtgtttctcaaatgaccgcgctggcaatggctttagggctggcttgcgcttcttcgtgggccgctgaactggcgaagcctcttacacttgaccagcttcaacaacaaaatggcaaagcgattgatactcgccccagcgcgttttataacggctggccacaaaccttaaatggcccttccggtcatgaacctgccgccttaaacctctctgctagctggctcgacaaaatgagcaccgaacagctcaacgagtggatcaagcaacataacctgaaagccgatgccccggtggcgctgtacggtaatgacaaagatgtcgacgccgtcaaaacgcgactgcaaaaagcaggttttacgcatatctccatcctgagtgacgcgctaagcgaaccttcccgtctgcaaaaactgccgcactttgaacagctggtatatccgcagtggctgcataacctgcaacaaggtaaagaggttacggcgaaacctgccggtgactggaaagtcattgaagcggcctggggcgctccaaaattttaccttatcagccatattcccggcgctgactacatcgacaccaacgaagtggaaagcgaaccgctgtggaacaaagtttctgatgaacaactgaaagcgatgctggcaaaacacggcattcgccatgacaccacggtcattctgtacgggcgtgacgtatacgctgcagcgcgtgtggcgcaaattatgctttatgccggcgtgaaagatgtgcgcctgctggacggaggctggcaaacctggtccgacgcgggtctgcccgttgagcgcggaacgccaccgaaagtgaaagcggaaccggatttcggcgtgaagatcccggcacaaccgcaactgatgcttgatatggaacaagcgcgtggactgctgcatcgccaggatgcatcgctggtgagcattcgttcgtggccagaatttatcggtacgaccagcggttacagctatattaaaccaaaaggtgaaatagccggagcacgttggggacacgcaggtagcgactcgacgcatatggaagatttccataacccggatggcaccatgcgcagcgccgatgatataaccgctatgtggaaagcatggaatatcaaaccagatcagcaagtttcattctactgcggcactggctggcgcgcgtcagaaacctttatgtacgcacgcgcaatgggctggaataacgtctccgtttacgacggtggctggtacgaatggagcagcgatccaaaaaatccggtagcaaccggtgaacgcggcccggacagcagtaaataa

SEQ ID NO: 13 - DNA, 30 bp, Artificial Sequence
  MsHisMT forward primer
gtgaaaggacgccatatgacgctctcactg

SEQ ID NO: 14 - DNA, 31 bp, Artificial Sequence
  MsHisMT reverse primer
cactgctgctcgagcatcaccgcaccgccag

SEQ ID NO: 15 - DNA, 30 bp, Artificial Sequence
  EcHerS forward primer
ctcaaaactaccatggcgggattttcgatg

SEQ ID NO: 16 - DNA, 31 bp, Artificial Sequence
  EcHerS reverse primer
gacgctgaagtcgctcgagcgtcagtaattg